European Patent Specification EP 3 765 478 B1, published July 24, 2024. Title: METHODS OF QUANTIFYING RNA AND DNA VARIANTS THROUGH SEQUENCING EMPLOYING PHOSPHOROTHIOATES. Applicant: MASSACHUSETTS INSTITUTE OF TECHNOLOGY. Application PCT/US2019/013714. The sequence listing filed with the application follows.

SEQUENCE LISTING (22 sequences)

SEQ ID NO: 1 - DNA, 20 bp, Artificial Sequence
  Synthetic Polynucleotide
  misc_feature (1)..(2): n is a, c, g, or t
  misc_feature (20)..(20): dideoxycytidine
nncactcgggcaccaaggac

SEQ ID NO: 2 - DNA, 19 bp, Artificial Sequence
  Synthetic Polynucleotide
  misc_feature (1)..(2): n is a, c, g, or t
  misc_feature (19)..(19): dideoxycytidine
nncactcgggcaccaggac

SEQ ID NO: 3 - DNA, 18 bp, Artificial Sequence
  Synthetic Polynucleotide
  misc_feature (1)..(2): phosphothioate linkage between the indicated residues
  misc_feature (2)..(3): phosphothioate linkage between the indicated residues
  misc_feature (3)..(4): phosphothioate linkage between the indicated residues
  misc_feature (4)..(5): phosphothioate linkage between the indicated residues
  misc_feature (5)..(6): phosphothioate linkage between the indicated residues
  misc_feature (6)..(7): phosphothioate linkage between the indicated residues
gtccttggtgcccgagtg

SEQ ID NO: 4 - DNA, 40 bp, Artificial Sequence
  Synthetic Polynucleotide
  misc_feature (23)..(28): n is a, c, g, or t
  misc_feature (40)..(40): modified by propyl spacer
tgaagagcctagtcgctgttcannnnnnctgcccatagag

SEQ ID NO: 5 - DNA, 41 bp, Artificial Sequence
  Synthetic Polynucleotide
  misc_feature (23)..(28): n is a, c, g, or t
  misc_feature (41)..(41): modified by propyl spacer
tgaagagcctagtcgctgttcannnnnnctgcccatagagc

SEQ ID NO: 6 - DNA, 90 bp, Artificial Sequence
  Synthetic Polynucleotide
  misc_feature (30)..(35): n is a, c, g, or t; barcode sequence
aatgatacggcgaccaccgagatctacacnnnnnnacactctttccctacacgacgctcttccgatcttgaacagcgactaggctcttca

SEQ ID NO: 7 - DNA, 85 bp, Artificial Sequence
  Synthetic Polynucleotide
  misc_feature (25)..(30): n is a, c, g, or t; barcode sequence
caagcagaagacggcatacgagatnnnnnncggtctcggcattcctgctgaaccgctcttccgatctgtccttggtgcccgagtg

SEQ ID NO: 8 - DNA, 63 bp, Artificial Sequence
  Synthetic Polynucleotide
tgaccccggtctacacattcgggagggcatagcatcaatagatgtgctgcccctcagtccgtt

SEQ ID NO: 9 - DNA, 63 bp, Artificial Sequence
  Synthetic Polynucleotide
aacggactgaggggcagcacatctattgatgctatgccctcccgaatgugtagaccggggtca

SEQ ID NO: 10 - DNA, 49 bp, Artificial Sequence
  Synthetic Polynucleotide
acattcgggagggcatagcatcaatagatgtgctgcccctcagtccgtt

SEQ ID NO: 11 - DNA, 49 bp, Artificial Sequence
  Synthetic Polynucleotide
aacggactgaggggcagcacatctattgatgctatgccctcccgaatgu

SEQ ID NO: 12 - DNA, 63 bp, Artificial Sequence
  Synthetic Polynucleotide
  misc_feature (49)..(49): n is an AP site
aacggactgaggggcagcacatctattgatgctatgccctcccgaatgngtagaccggggtca

SEQ ID NO: 13 - DNA, 49 bp, Artificial Sequence
  Synthetic Polynucleotide
  misc_feature (49)..(49): n is an AP site
aacggactgaggggcagcacatctattgatgctatgccctcccgaatgn

SEQ ID NO: 14 - DNA, 63 bp, Artificial Sequence
  Synthetic Polynucleotide
tgaccccggtctacccattcgggagggcatagcatcaatagatgtgctgcccctcagtccgtt

SEQ ID NO: 15 - DNA, 63 bp, Artificial Sequence; identical to SEQ ID NO: 12
  Synthetic Polynucleotide
  misc_feature (49)..(49): n is inosine

SEQ ID NO: 16 - DNA, 49 bp, Artificial Sequence
  Synthetic Polynucleotide
  misc_feature (1)..(1): n is a or c
ncattcgggagggcatagcatcaatagatgtgctgcccctcagtccgtt

SEQ ID NO: 17 - DNA, 49 bp, Artificial Sequence; identical to SEQ ID NO: 13
  Synthetic Polynucleotide
  misc_feature (49)..(49): n is inosine

SEQ ID NO: 18 - DNA, 63 bp, Artificial Sequence
  Synthetic Polynucleotide
tgaccccggtctactcattcgggagggcatagcatcaatagatgtgctgcccctcagtccgtt

SEQ ID NO: 19 - DNA, 63 bp, Artificial Sequence
  Synthetic Polynucleotide
aacggactgaggggcagcacatctattgatgctatgccctcccgaatgagtagaccggggtca

SEQ ID NO: 20 - DNA, 49 bp, Artificial Sequence
  Synthetic Polynucleotide
tcattcgggagggcatagcatcaatagatgtgctgcccctcagtccgtt

SEQ ID NO: 21 - DNA, 49 bp, Artificial Sequence
  Synthetic Polynucleotide
aacggactgaggggcagcacatctattgatgctatgccctcccgaatga

SEQ ID NO: 22 - DNA, 36 bp, Artificial Sequence
  Synthetic Polynucleotide
ttcggcaaacggcattccgtctacccaacacgaagc